European Patent Specification EP 3 417 872 B1, published January 24, 2024. Title: Agent for improving intestinal flora. Applicant: Amano Enzyme Inc. Hiroshima University. The sequence listing filed with the application follows.

SEQUENCE LISTING (1 sequence)

SEQ ID NO: 1 - protein, 323 aa, Aspergillus oryzae
ASGHGTVVTSPEPNDIEYLTPVNIGGTTLNLDFDTGSADLWVFSEELPKSEQTGHDVYKPSGNASKIAGASWDISYGDGSSASGDVYQDTVTVGGVTAQGQAVEAASKISDQFVQDKNNDGLLGLAFSSINTVKPKPQTTFFDTVKDQLDAPLFAVTLKYHAPGSYDFGFIDKSKFTGELAYADVDDSQGFWQFTADGYSVGKGDAQKAPITGIADTGTTLVMLDDEIVDAYYKQVQGAKNDASAGGYVFPCETELPEFTVVIGSYNAVIPGKHINYAPLQEGSSTCVGGIQSNSGLGLSILGDVFLKSQYVVFDSQGPRLGF